European Patent Application EP 4 570 909 A1, published June 18, 2025. Title: 光响应型核酸适配体、光启动DNA聚合酶及应用. Applicant: Sun Yat-Sen University. The sequence listing filed with the application follows.

SEQUENCE LISTING (39 sequences)

SEQ ID NO: 1 - DNA, 15 bp, synthetic construct
  source 1..15: mol_type = other DNA
gggtgggtgggtggg

SEQ ID NO: 2 - protein, 64 aa, synthetic construct
HPGHLKGREIGMWYAKKQGQKNKGTGSGAGTGSGAGTGSGAHPGHLKGREIGMWYAKKQGQKNK

SEQ ID NO: 3 - protein, 588 aa, synthetic construct
AAEGEKPLEEMEFAIVDVITEEMLADKAALVVEVMEENYHDAPIVGIALVNEHGRFFMRPETALADSQFLAWLADETKKKSMFDAKRAVVALKWKGIELRGVAFDLLLAAYLLNPAQDAGDIAAVAKMKQYEAVRSDEAVYGKGAKRSLPDEQTLAEHLVRKAAAIWALEQPFMDDLRNNEQDQLLTKLEQPLAAILAEMEFTGVNVDTKRLEQMGSELAEQLRAIEQRIYELAGQEFNINSPKQLGVILFEKLQLPVLKKTKTGYSTSADVLEKLAPHHEIVENILHYRQLGKLQSTYIEGLLKVVRPDTGKVHTMFNQALTQTGRLSSAEPNLQNIPIRLEEGRKIRQAFVPSEPDWLIFAADYSQIELRVLAHIADDDNLIEAFQRDLDIHTKTAMDIFHVSEEEVTANMRRQAKAVNFGIVYGISDYGLAQNLNITRKEAAEFIERYFASFPGVKQYMENIVQEAKQKGYVTTLLHRRRYLPDITSRNFNVRSFAERTAMNTPIQGSAADIIKKAMIDLAARLKEEQLQARLLLQVHDELILEAPKEEIERLCELVPEVMEQAVTLRVPLKVDYHYGPTWYDAK

SEQ ID NO: 4 - protein, 585 aa, synthetic construct
MDQSLEDINVKTVTDVTSDILVSPSAFVVEQIGDNYHEEPILGFSIVNETGAYFIPKDIAVESEVFKEWVENDEQKKWVFDSKRAVVALRWQGIELKGAEFDTLLAAYIINPGNSYDDVASVAKDYGLHIVSSDESVYGKGAKRAVPSEDVLSEHLGRKALAIQSLREKLVQELENNDQLELFEELEMPLALILGEMESTGVKVDVDRLKRMGEELGAKLKEYEEKIHEIAGEPFNINSPKQLGVILFEKIGLPVVKKTKTGYSTSADVLEKLADKHDIVDYILQYRQIGKLQSTYIEGLLKVTRPDSHKVHTRFNQALTQTGRLSSTDPNLQNIPIRLEEGRKIRQAFVPSEKDWLIFAADYSQIELRVLAHISKDENLIEAFTNDMDIHTKTAMDVFHVAKDEVTSAMRRQAKAVNFGIVYGISDYGLSQNLGITRKEAGAFIDRYLESFQGVKAYMEDSVQEAKQKGYVTTLMHRRRYIPELTSRNFNIRSFAERTAMNTPIQGSAADIIKKAMIDMAAKLKEKQLKARLLLQVHDELIFEAPKEEIEILEKLVPEVMEHALALDVPLKVDFASGPSWYDAK

SEQ ID NO: 5 - protein, 590 aa, synthetic construct
IEGRISHHPGHLKGREIGMWYAKKQGQKNKAKKWKWKSLLHEFGLLESPKALEEAPWPPPEGAFVGFVLSRKEPMWADLLALAAARGGRVHRAPEPYKALRDLKEARGLLAKDLSVLALREGLGLPPGDDPMLLAYLLDPSNTTPEGVARRYGGEWTEEAGERAALSERLFANLWGRLEGEERLLWLYREVERPLSAVLAHMEATGVRLDVAYLRALSLEVAEEIARLEAEVFRLAGHPFNLNSRDQLERVLFDELGLPAIGKTEKTGKRSTSAAVLEALREAHPIVEKILQYRELTKLKSTYIDPLPDLIHPRTGRLHTRFNQTATATGRLSSSDPNLQNIPVRTPLGQRIRRAFIAEEGWLLVALDYSQIELRVLAHLSGDENLIRVFQEGRDIHTETASWMFGVPREAVDPLMRRAAKTINFGVLYGMSAHRLSQELAIPYEEAQAFIERYFQSFPKVRAWIEKTLEEGRRRGYVETLFGRRRYVPDLEARVKSVREAAERMAFNMPVQGTAADLMKLAMVKLFPRLEEMGARMLLQVHDELVLEAPKERAEAVARLAKEVMEGVYPLAVPLEVEVGIGEDWLSAKE

SEQ ID NO: 6 - DNA, 30 bp, synthetic construct
  source 1..30: mol_type = other DNA
cgcagaccagttttctggtctgcgtttttt

SEQ ID NO: 7 - DNA, 17 bp, synthetic construct
  source 1..17: mol_type = other DNA
tgggtgggtgggtgggt

SEQ ID NO: 8 - DNA, 17 bp, synthetic construct
  source 1..17: mol_type = other DNA
ccagcctgcggcgagtg

SEQ ID NO: 9 - DNA, 67 bp, synthetic construct
  source 1..67: mol_type = other DNA
tctattacattctaagagttagagttagggtctactcttcttctcttcttcactcgccgcaggctgg

SEQ ID NO: 10 - DNA, 12 bp, synthetic construct
  source 1..12: mol_type = other DNA
cgcagaccagtt

SEQ ID NO: 11 - DNA, 35 bp, synthetic construct
  source 1..35: mol_type = other DNA
ttctggtctgcgtttttttgggtgggtgggtgggt

SEQ ID NO: 12 - DNA, 34 bp, synthetic construct
  source 1..34: mol_type = other DNA
cgcagaccagttttctggtctgcgtttttttggg

SEQ ID NO: 13 - DNA, 13 bp, synthetic construct
  source 1..13: mol_type = other DNA
tgggtgggtgggt

SEQ ID NO: 14 - DNA, 38 bp, synthetic construct
  source 1..38: mol_type = other DNA
cgcagaccagttttctggtctgcgtttttttgggtggg

SEQ ID NO: 15 - DNA, 42 bp, synthetic construct
  source 1..42: mol_type = other DNA
cgcagaccagttttctggtctgcgtttttttgggtgggtggg

SEQ ID NO: 16 - DNA, 24 bp, synthetic construct
  source 1..24: mol_type = other DNA
agaccagttttctggtcttttttt

SEQ ID NO: 17 - DNA, 17 bp, synthetic construct
  source 1..17: mol_type = other DNA
tgggtgggtgggtgggt

SEQ ID NO: 18 - DNA, 30 bp, synthetic construct; identical to SEQ ID NO: 6
  source 1..30: mol_type = other DNA

SEQ ID NO: 19 - DNA, 17 bp, synthetic construct
  source 1..17: mol_type = other DNA
tgggtgggtgggtgggt

SEQ ID NO: 20 - DNA, 36 bp, synthetic construct
  source 1..36: mol_type = other DNA
cgacgcagaccagttttctggtctgcgtcgtttttt

SEQ ID NO: 21 - DNA, 17 bp, synthetic construct
  source 1..17: mol_type = other DNA
tgggtgggtgggtgggt

SEQ ID NO: 22 - DNA, 42 bp, synthetic construct
  source 1..42: mol_type = other DNA
ccacgacgcagaccagttttctggtctgcgtcgtggtttttt

SEQ ID NO: 23 - DNA, 17 bp, synthetic construct
  source 1..17: mol_type = other DNA
tgggtgggtgggtgggt

SEQ ID NO: 24 - DNA, 22 bp, synthetic construct
  source 1..22: mol_type = other DNA
gctgctgatgaagatgatgacg

SEQ ID NO: 25 - DNA, 23 bp, synthetic construct
  source 1..23: mol_type = other DNA
tgtaaaggctcacagacccaata

SEQ ID NO: 26 - DNA, 22 bp, synthetic construct
  source 1..22: mol_type = other DNA
gccctttcctatgcttagatgc

SEQ ID NO: 27 - DNA, 24 bp, synthetic construct
  source 1..24: mol_type = other DNA
ttactttaattggactgccttcgt

SEQ ID NO: 28 - DNA, 22 bp, synthetic construct
  source 1..22: mol_type = other DNA
gccatttgggaatttaggtagg

SEQ ID NO: 29 - DNA, 23 bp, synthetic construct
  source 1..23: mol_type = other DNA
ccgttcttaaagataactggtgc

SEQ ID NO: 30 - DNA, 22 bp, synthetic construct
  source 1..22: mol_type = other DNA
tgtgccagttcttgggtttgtt

SEQ ID NO: 31 - DNA, 25 bp, synthetic construct
  source 1..25: mol_type = other DNA
caggaccttgaagtgattatttgtg

SEQ ID NO: 32 - DNA, 26 bp, synthetic construct
  source 1..26: mol_type = other DNA
tgtccctttgttctgaagatttagtg

SEQ ID NO: 33 - DNA, 21 bp, synthetic construct
  source 1..21: mol_type = other DNA
ggctgggtgttaggattacgg

SEQ ID NO: 34 - DNA, 24 bp, synthetic construct
  source 1..24: mol_type = other DNA
catgaagttgctgtattgggattt

SEQ ID NO: 35 - DNA, 25 bp, synthetic construct
  source 1..25: mol_type = other DNA
agcgttcatagcagtcaacaagtag

SEQ ID NO: 36 - DNA, 26 bp, synthetic construct
  source 1..26: mol_type = other DNA
tggagtaggacctgattgtagtattg

SEQ ID NO: 37 - DNA, 22 bp, synthetic construct
  source 1..22: mol_type = other DNA
cgaaccttcatgcacctctttg

SEQ ID NO: 38 - DNA, 23 bp, synthetic construct
  source 1..23: mol_type = other DNA
ttttcgtggcttcagtagattcc

SEQ ID NO: 39 - DNA, 21 bp, synthetic construct
  source 1..21: mol_type = other DNA
tgggcagcatggctagtatct